European Patent Application EP 4 725 969 A1, published April 15, 2026. Title: 抗HER2互补性双特异抗体-药物偶联物及其制备方法和用途. Applicant: 徕特康（苏州）生物制药有限公司. The sequence listing filed with the application follows.

SEQUENCE LISTING (234 sequences)

SEQ ID NO: 1 - protein, 117 aa, Mus musculus
EVKIEESGGGLVKPGGSLKLSCAASGFTYSSYGMSWVRQTPEKRLEWVASISGGGSYTKYPDSVKGRFTISRDNAKNHLYLQMSSLRSEDTALYYCARDYAGFFDVWGAGTTVTVSS

SEQ ID NO: 2 - protein, 112 aa, Mus musculus
DVVLTQTPLSLPVSLGDQASISCRSSQSLVHSNGNTYLHWYLQKPGQSPKLLIYKVSNRFSGVPDRFSGSGSGTDFTLKISRVEAEDLGVYFCSQSTHVPYTFGGGTKLEIK

SEQ ID NO: 3 - protein, 119 aa, Mus musculus
QIQLAQSGPELKKPGETVKISCKASGYTFTDYSMHWVKQAPGKYLKWMGWINTETGEPTYADDFKGRFAFSLETSANTAYLQINNLKNEDTATYFCVRVGRYDYAMDYWGQGTSVTVSS

SEQ ID NO: 4 - protein, 107 aa, Mus musculus
DIVMTQSHKFMSTSVGDRVSITCKASQDVYTAVAWYQQKPGQSPKLLINSASYRYTGVPDRFTGSGSGTDFTFTISSVQAEDLAVYYCQQHYSTPPTFGGGTKLEIK

SEQ ID NO: 5 - protein, 119 aa, Mus musculus
EVQLQQSGPELVKPGASVKIPCKASGYTFTDYNMDWVKQSHGKSLEWIGDINPNNGGTIYNQKFKGKATLTVDKSSSTAYMELRSLTSEDTAVYYCARYGSGYGGFAYWGQGTLVTVSS

SEQ ID NO: 6 - protein, 108 aa, Mus musculus
DIVLTQSPTTMAASPGEKITITCSASSSISSNYLHWYQQKPGFSPKLLIYRTSNLASGVPARFSGSGSGTSYSLTIGTMEAEDVATYYCQQGSSIPRTFGGGTKLEIK

SEQ ID NO: 7 - protein, 120 aa, Mus musculus
QIQLQQSGAELMKPGASVKISCKTTGYTFSNYWIEWVKQRPGHGLEWIGEILPGGDSANYNEIFKGKATFTADTSSNTAYMQLSSLTSEDSAVYFCARGGGNYPYYFDSWGQGTTLTVSS

SEQ ID NO: 8 - protein, 107 aa, Mus musculus
DILLTQSHKFMSTSVGDRVSITCKASQDVGTAVAWYQQKPGQSPKLLIYWASTRHTGVPDRFTGSGSGTDFTLTISNVQSEDLADYFCQQYSSYPRTFGGGTKLEIK

SEQ ID NO: 9 - protein, 120 aa, Mus musculus
QAYLQQSGAELMKPGASVKISCKATGYTFSNYWIEWVRQRPGHGLEWIGEILPGSDTSKNNEIFKGKATFTADTSSSTAYMQLSSLTSEDSAVYYCARGGNNYPYYFDYWGQGTTLTVSS

SEQ ID NO: 10 - protein, 107 aa, Mus musculus
DILMTQSHKFMSTSVGDRVSITCKASQDVGTAVAWYQQKPGQSPKLLIYWASTRHTGVPDRFTGSGSGTDFTLTISNVQSEDLADYFCQQYSSYPWTFGGGTKLEIK

SEQ ID NO: 11 - protein, 5 aa, Mus musculus
SYGMS

SEQ ID NO: 12 - protein, 5 aa, synthetic construct
  source 1..5: note; note (original language) = 人源化抗体hu2117-HK-Mu38和39的HCDR1
NYGMS

SEQ ID NO: 13 - protein, 5 aa, synthetic construct
  source 1..5: note; note (original language) = 人源化抗体hu2117-HK-Mu40的HCDR1
DYGMS

SEQ ID NO: 14 - protein, 17 aa, Mus musculus
SISGGGSYTKYPDSVKG

SEQ ID NO: 15 - protein, 17 aa, synthetic construct
  source 1..17: note; note (original language) = 人源化抗体hu2117-HK-Mu08的HCDR2
SISGGGSYTKYADSVKG

SEQ ID NO: 16 - protein, 17 aa, synthetic construct
  source 1..17: note; note (original language) = 人源化抗体hu2117-HK-Mu09的HCDR2
SISGGGSYTKYGDSVKG

SEQ ID NO: 17 - protein, 17 aa, synthetic construct
  source 1..17: note; note (original language) = 人源化抗体hu2117-HK-Mu10的HCDR2
SISGGGSYTKYVDSVKG

SEQ ID NO: 18 - protein, 17 aa, synthetic construct
  source 1..17: note; note (original language) = 人源化抗体hu2117-HK-Mu14的HCDR2
SISGGGSYTKYPGSVKG

SEQ ID NO: 19 - protein, 17 aa, synthetic construct
  source 1..17: note; note (original language) = 人源化抗体hu2117-HK-Mu41的HCDR2
SISGGGNYAKYPDSVKG

SEQ ID NO: 20 - protein, 17 aa, synthetic construct
  source 1..17: note; note (original language) = 人源化抗体hu2117-HK-Mu42的HCDR2
SISGSGSYTKYPDSVKG

SEQ ID NO: 21 - protein, 17 aa, synthetic construct
  source 1..17: note; note (original language) = 人源化抗体hu2117-HK201、HK203的HCDR2
SISGGGNYAKYVDSVKG

SEQ ID NO: 22 - protein, 17 aa, synthetic construct
  source 1..17: note; note (original language) = 人源化抗体hu2117-HK301的HCDR2
SISGGGNYAKYVGSVKG

SEQ ID NO: 23 - protein, 17 aa, synthetic construct
  source 1..17: note; note (original language) = 人源化抗体hu2117-HK303的HCDR2
SISGGGNYAKYVESVKG

SEQ ID NO: 24 - protein, 17 aa, synthetic construct
  source 1..17: note; note (original language) = 人源化抗体hu2117-HK304的HCDR2
SISGGGNYAKYVPSVKG

SEQ ID NO: 25 - protein, 17 aa, synthetic construct
  source 1..17: note; note (original language) = 人源化抗体hu2117-HK305的HCDR2
SISGGGNYAKYVQSVKG

SEQ ID NO: 26 - protein, 17 aa, synthetic construct
  source 1..17: note; note (original language) = 人源化抗体hu2117-HK306的HCDR2
SISGGGNYAKYVRSVKG

SEQ ID NO: 27 - protein, 17 aa, synthetic construct
  source 1..17: note; note (original language) = 人源化抗体hu2117-HK309的HCDR2
SISGGGNYAKYVDKVKG

SEQ ID NO: 28 - protein, 17 aa, synthetic construct
  source 1..17: note; note (original language) = 人源化抗体hu2117-HK310的HCDR2
SISGGGNYAKYVDNVKG

SEQ ID NO: 29 - protein, 17 aa, synthetic construct
  source 1..17: note; note (original language) = 人源化抗体hu2117-HK304-04的HCDR2
SISGGGSYTKYPESVKG

SEQ ID NO: 30 - protein, 17 aa, synthetic construct
  source 1..17: note; note (original language) = 人源化抗体hu2117-HK304-05的HCDR2
SISGGGSYTKYPDKVKG

SEQ ID NO: 31 - protein, 17 aa, synthetic construct
  source 1..17: note; note (original language) = 人源化抗体hu2117-HK304-06的HCDR2
SISGGGSYTKYVDKVKG

SEQ ID NO: 32 - protein, 8 aa, Mus musculus
DYAGFFDV

SEQ ID NO: 33 - protein, 8 aa, synthetic construct
  source 1..8: note; note (original language) = 人源化抗体hu2117-HK-Mu45的HCDR3
DYIGFFDV

SEQ ID NO: 34 - protein, 8 aa, synthetic construct
  source 1..8: note; note (original language) = 人源化抗体hu2117-HK-Mu46的HCDR3
DYNGFFDV

SEQ ID NO: 35 - protein, 8 aa, synthetic construct
  source 1..8: note; note (original language) = 人源化抗体hu2117-HK-Mu48的HCDR3
DYRGFFDV

SEQ ID NO: 36 - protein, 8 aa, synthetic construct
  source 1..8: note; note (original language) = 人源化抗体hu2117-HK-Mu49的HCDR3
DYSGFFDV

SEQ ID NO: 37 - protein, 8 aa, synthetic construct
  source 1..8: note; note (original language) = HCDR3
DYVGFFDV

SEQ ID NO: 38 - protein, 16 aa, Mus musculus
RSSQSLVHSNGNTYLH

SEQ ID NO: 39 - protein, 16 aa, synthetic construct
  source 1..16: note; note (original language) = 人源化抗体hu2117-HK-Mu23的LCDR1
RSSQSLVHSNANTYLH

SEQ ID NO: 40 - protein, 16 aa, synthetic construct
  source 1..16: note; note (original language) = 人源化抗体hu2117-HK-Mu24的LCDR1
RSSQSLVHSNINTYLH

SEQ ID NO: 41 - protein, 16 aa, synthetic construct
  source 1..16: note; note (original language) = 人源化抗体hu2117-HK-Mu25的LCDR1
RSSQSLVHSNSNTYLH

SEQ ID NO: 42 - protein, 16 aa, synthetic construct
  source 1..16: note; note (original language) = LCDR1
RSSQSLVHSNRNTYLH

SEQ ID NO: 43 - protein, 16 aa, synthetic construct
  source 1..16: note; note (original language) = 人源化抗体hu2117-HK-Mu28的LCDR1
RSSQSLVHSNTNTYLH

SEQ ID NO: 44 - protein, 16 aa, synthetic construct
  source 1..16: note; note (original language) = 人源化抗体hu2117-HK-Mu29的LCDR1
RSSQSLLHSNGNTYLH

SEQ ID NO: 45 - protein, 16 aa, synthetic construct
  source 1..16: note; note (original language) = 人源化抗体hu2117-HK-Mu32的LCDR1
RSSQSLVSSNGNTYLH

SEQ ID NO: 46 - protein, 7 aa, Mus musculus
KVSNRFS

SEQ ID NO: 47 - protein, 7 aa, synthetic construct
  source 1..7: note; note (original language) = 人源化抗体hu2117-HK-Mu11的LCDR2
KVSNRDS

SEQ ID NO: 48 - protein, 7 aa, synthetic construct
  source 1..7: note; note (original language) = 人源化抗体hu2117-HK-Mu12的LCDR2
KVSNRPS

SEQ ID NO: 49 - protein, 9 aa, Mus musculus
SQSTHVPYT

SEQ ID NO: 50 - protein, 9 aa, synthetic construct
  source 1..9: note; note (original language) = 人源化抗体hu2117-HK-Mu34的LCDR3
QQSTHVPYT

SEQ ID NO: 51 - protein, 9 aa, synthetic construct
  source 1..9: note; note (original language) = 人源化抗体hu2117-HK-Mu37的LCDR3
SQSTHVPWT

SEQ ID NO: 52 - protein, 117 aa, synthetic construct
  source 1..117: note; note (original language) = VH
EVQLVESGGGLVQPGGSLRLSCAASGFTYSSYGMSWVRQAPGKGLEWVASISGGGSYTKYPDSVKGRFTISRDNSKNTLYLQMNSLRAEDTAVYYCARDYAGFFDVWGQGTLVTVSS

SEQ ID NO: 53 - protein, 117 aa, synthetic construct
  source 1..117: note; note (original language) = 人源化抗体hu2117-HK-Mu05的VH
EVQLVESGGGLVQPGGSLRLSCAASGFTFSSYGMSWVRQAPGKGLEWVASISGGGSYTKYPDSVKGRFTISRDNSKNTLYLQMNSLRAEDTAVYYCARDYAGFFDVWGQGTLVTVSS

SEQ ID NO: 54 - protein, 117 aa, synthetic construct
  source 1..117: note; note (original language) = 人源化抗体hu2117-HK-Mu06的VH
EVQLVESGGGLVQPGGSLRLSCAASGFTYSSYGMSWVRQAPGKGLEWVSSISGGGSYTKYPDSVKGRFTISRDNSKNTLYLQMNSLRAEDTAVYYCARDYAGFFDVWGQGTLVTVSS

SEQ ID NO: 55 - protein, 117 aa, synthetic construct
  source 1..117: note; note (original language) = 人源化抗体hu2117-H1K1-Mu08的VH
EVQLVESGGGLVQPGGSLRLSCAASGFTYSSYGMSWVRQAPGKGLEWVASISGGGSYTKYADSVKGRFTISRDNSKNTLYLQMNSLRAEDTAVYYCARDYAGFFDVWGQGTLVTVSS

SEQ ID NO: 56 - protein, 117 aa, synthetic construct
  source 1..117: note; note (original language) = 人源化抗体hu2117-H1K1-Mu09的VH
EVQLVESGGGLVQPGGSLRLSCAASGFTYSSYGMSWVRQAPGKGLEWVASISGGGSYTKYGDSVKGRFTISRDNSKNTLYLQMNSLRAEDTAVYYCARDYAGFFDVWGQGTLVTVSS

SEQ ID NO: 57 - protein, 117 aa, synthetic construct
  source 1..117: note; note (original language) = 人源化抗体hu2117-H1K1-Mu10的VH
EVQLVESGGGLVQPGGSLRLSCAASGFTYSSYGMSWVRQAPGKGLEWVASISGGGSYTKYVDSVKGRFTISRDNSKNTLYLQMNSLRAEDTAVYYCARDYAGFFDVWGQGTLVTVSS

SEQ ID NO: 58 - protein, 117 aa, synthetic construct
  source 1..117: note; note (original language) = 人源化抗体hu2117-H1K1-Mu14的VH
EVQLVESGGGLVQPGGSLRLSCAASGFTYSSYGMSWVRQAPGKGLEWVASISGGGSYTKYPGSVKGRFTISRDNSKNTLYLQMNSLRAEDTAVYYCARDYAGFFDVWGQGTLVTVSS

SEQ ID NO: 59 - protein, 117 aa, synthetic construct
  source 1..117: note; note (original language) = 人源化抗体hu2117-H1K1-Mu38的VH
EVQLVESGGGLVQPGGSLRLSCAASGFTYNNYGMSWVRQAPGKGLEWVASISGGGSYTKYPDSVKGRFTISRDNSKNTLYLQMNSLRAEDTAVYYCARDYAGFFDVWGQGTLVTVSS

SEQ ID NO: 60 - protein, 117 aa, synthetic construct
  source 1..117: note; note (original language) = 人源化抗体hu2117-H1K1-Mu39的VH
EVQLVESGGGLVQPGGSLRLSCAASGFTYSNYGMSWVRQAPGKGLEWVASISGGGSYTKYPDSVKGRFTISRDNSKNTLYLQMNSLRAEDTAVYYCARDYAGFFDVWGQGTLVTVSS

SEQ ID NO: 61 - protein, 117 aa, synthetic construct
  source 1..117: note; note (original language) = 人源化抗体hu2117-H1K1-Mu40的VH
EVQLVESGGGLVQPGGSLRLSCAASGFTYSDYGMSWVRQAPGKGLEWVASISGGGSYTKYPDSVKGRFTISRDNSKNTLYLQMNSLRAEDTAVYYCARDYAGFFDVWGQGTLVTVSS

SEQ ID NO: 62 - protein, 117 aa, synthetic construct
  source 1..117: note; note (original language) = 人源化抗体hu2117-H1K1-Mu41的VH
EVQLVESGGGLVQPGGSLRLSCAASGFTYSSYGMSWVRQAPGKGLEWVASISGGGNYAKYPDSVKGRFTISRDNSKNTLYLQMNSLRAEDTAVYYCARDYAGFFDVWGQGTLVTVSS

SEQ ID NO: 63 - protein, 117 aa, synthetic construct
  source 1..117: note; note (original language) = 人源化抗体hu2117-H1K1-Mu42的VH
EVQLVESGGGLVQPGGSLRLSCAASGFTYSSYGMSWVRQAPGKGLEWVASISGSGSYTKYPDSVKGRFTISRDNSKNTLYLQMNSLRAEDTAVYYCARDYAGFFDVWGQGTLVTVSS

SEQ ID NO: 64 - protein, 117 aa, synthetic construct
  source 1..117: note; note (original language) = 人源化抗体hu2117-H1K1-Mu45的VH
EVQLVESGGGLVQPGGSLRLSCAASGFTYSSYGMSWVRQAPGKGLEWVASISGGGSYTKYPDSVKGRFTISRDNSKNTLYLQMNSLRAEDTAVYYCARDYIGFFDVWGQGTLVTVSS

SEQ ID NO: 65 - protein, 117 aa, synthetic construct
  source 1..117: note; note (original language) = 人源化抗体hu2117-H1K1-Mu46的VH
EVQLVESGGGLVQPGGSLRLSCAASGFTYSSYGMSWVRQAPGKGLEWVASISGGGSYTKYPDSVKGRFTISRDNSKNTLYLQMNSLRAEDTAVYYCARDYNGFFDVWGQGTLVTVSS

SEQ ID NO: 66 - protein, 117 aa, synthetic construct
  source 1..117: note; note (original language) = 人源化抗体hu2117-H1K1-Mu48的VH
EVQLVESGGGLVQPGGSLRLSCAASGFTYSSYGMSWVRQAPGKGLEWVASISGGGSYTKYPDSVKGRFTISRDNSKNTLYLQMNSLRAEDTAVYYCARDYRGFFDVWGQGTLVTVSS

SEQ ID NO: 67 - protein, 117 aa, synthetic construct
  source 1..117: note; note (original language) = 人源化抗体hu2117-H1K1-Mu49的VH
EVQLVESGGGLVQPGGSLRLSCAASGFTYSSYGMSWVRQAPGKGLEWVASISGGGSYTKYPDSVKGRFTISRDNSKNTLYLQMNSLRAEDTAVYYCARDYSGFFDVWGQGTLVTVSS

SEQ ID NO: 68 - protein, 117 aa, synthetic construct
  source 1..117: note; note (original language) = 人源化抗体hu2117-H1K1-Mu50、hu2117-HK202的VH
EVQLVESGGGLVQPGGSLRLSCAASGFTYSSYGMSWVRQAPGKGLEWVASISGGGSYTKYPDSVKGRFTISRDNSKNTLYLQMNSLRAEDTAVYYCARDYVGFFDVWGQGTLVTVSS

SEQ ID NO: 69 - protein, 117 aa, synthetic construct
  source 1..117: note; note (original language) = 人源化抗体hu2117-HK201的VH
EVQLVESGGGLVQPGGSLRLSCAASGFTYSSYGMSWVRQAPGKGLEWVASISGGGNYAKYVDSVKGRFTISRDNSKNTLYLQMNSLRAEDTAVYYCARDYAGFFDVWGQGTLVTVSS

SEQ ID NO: 70 - protein, 117 aa, synthetic construct
  source 1..117: note; note (original language) = 人源化抗体hu2117-HK203的VH
EVQLVESGGGLVQPGGSLRLSCAASGFTYSSYGMSWVRQAPGKGLEWVASISGGGNYAKYVDSVKGRFTISRDNSKNTLYLQMNSLRAEDTAVYYCARDYVGFFDVWGQGTLVTVSS

SEQ ID NO: 71 - protein, 117 aa, synthetic construct
  source 1..117: note; note (original language) = 人源化抗体hu2117-HK301的VH
EVQLVESGGGLVQPGGSLRLSCAASGFTYSSYGMSWVRQAPGKGLEWVASISGGGNYAKYVGSVKGRFTISRDNSKNTLYLQMNSLRAEDTAVYYCARDYVGFFDVWGQGTLVTVSS

SEQ ID NO: 72 - protein, 117 aa, synthetic construct
  source 1..117: note; note (original language) = 人源化抗体hu2117-HK303的VH
EVQLVESGGGLVQPGGSLRLSCAASGFTYSSYGMSWVRQAPGKGLEWVASISGGGNYAKYVESVKGRFTISRDNSKNTLYLQMNSLRAEDTAVYYCARDYVGFFDVWGQGTLVTVSS

SEQ ID NO: 73 - protein, 117 aa, synthetic construct
  source 1..117: note; note (original language) = 人源化抗体hu2117-HK304的VH
EVQLVESGGGLVQPGGSLRLSCAASGFTYSSYGMSWVRQAPGKGLEWVASISGGGNYAKYVPSVKGRFTISRDNSKNTLYLQMNSLRAEDTAVYYCARDYVGFFDVWGQGTLVTVSS

SEQ ID NO: 74 - protein, 117 aa, synthetic construct
  source 1..117: note; note (original language) = 人源化抗体hu2117-HK305的VH
EVQLVESGGGLVQPGGSLRLSCAASGFTYSSYGMSWVRQAPGKGLEWVASISGGGNYAKYVQSVKGRFTISRDNSKNTLYLQMNSLRAEDTAVYYCARDYVGFFDVWGQGTLVTVSS

SEQ ID NO: 75 - protein, 117 aa, synthetic construct
  source 1..117: note; note (original language) = 人源化抗体hu2117-HK306的VH
EVQLVESGGGLVQPGGSLRLSCAASGFTYSSYGMSWVRQAPGKGLEWVASISGGGNYAKYVRSVKGRFTISRDNSKNTLYLQMNSLRAEDTAVYYCARDYVGFFDVWGQGTLVTVSS

SEQ ID NO: 76 - protein, 117 aa, synthetic construct
  source 1..117: note; note (original language) = 人源化抗体hu2117-HK309的VH
EVQLVESGGGLVQPGGSLRLSCAASGFTYSSYGMSWVRQAPGKGLEWVASISGGGNYAKYVDKVKGRFTISRDNSKNTLYLQMNSLRAEDTAVYYCARDYVGFFDVWGQGTLVTVSS

SEQ ID NO: 77 - protein, 117 aa, synthetic construct
  source 1..117: note; note (original language) = 人源化抗体hu2117-HK310的VH
EVQLVESGGGLVQPGGSLRLSCAASGFTYSSYGMSWVRQAPGKGLEWVASISGGGNYAKYVDNVKGRFTISRDNSKNTLYLQMNSLRAEDTAVYYCARDYVGFFDVWGQGTLVTVSS

SEQ ID NO: 78 - protein, 117 aa, synthetic construct
  source 1..117: note; note (original language) = 人源化抗体hu2117-HK304-04的VH
QVQLVESGGGLVQPGGSLRLSCAASGFTYSSYGMSWVRQAPGKGLEWVASISGGGSYTKYPESVKGRFTISRDNSKNTLYLQMNSLRAEDTAVYYCARDYVGFFDVWGQGTLVTVSS

SEQ ID NO: 79 - protein, 117 aa, synthetic construct
  source 1..117: note; note (original language) = 人源化抗体hu2117-HK304-05的VH
QVQLVESGGGLVQPGGSLRLSCAASGFTYSSYGMSWVRQAPGKGLEWVASISGGGSYTKYPDKVKGRFTISRDNSKNTLYLQMNSLRAEDTAVYYCARDYVGFFDVWGQGTLVTVSS

SEQ ID NO: 80 - protein, 117 aa, synthetic construct
  source 1..117: note; note (original language) = 人源化抗体hu2117-HK304-06的VH
QVQLVESGGGLVQPGGSLRLSCAASGFTYSSYGMSWVRQAPGKGLEWVASISGGGSYTKYVDKVKGRFTISRDNSKNTLYLQMNSLRAEDTAVYYCARDYVGFFDVWGQGTLVTVSS

SEQ ID NO: 81 - protein, 112 aa, synthetic construct
  source 1..112: note; note (original language) = VL
DIQMTQSPSSLSASVGDRVTITCRSSQSLVHSNGNTYLHWYQQKPGKAPKLLIYKVSNRFSGVPSRFSGSGSGTDFTLTISSLQPEDFATYFCSQSTHVPYTFGQGTKVEIK

SEQ ID NO: 82 - protein, 112 aa, synthetic construct
  source 1..112: note; note (original language) = 人源化抗体hu2117-HK-Mu01的VL
DIQMTQSPSSLSASVGDRVTITCRSSQSLVHSNGNTYLHWYQQKPGKSPKLLIYKVSNRFSGVPSRFSGSGSGTDFTLTISSLQPEDFATYFCSQSTHVPYTFGQGTKVEIK

SEQ ID NO: 83 - protein, 112 aa, synthetic construct
  source 1..112: note; note (original language) = 人源化抗体hu2117-HK-Mu02的VL
DIQMTQSPSSLSASVGDRVTITCRSSQSLVHSNGNTYLHWYQQKPGKAPKLLIYKVSNRFSGVPSRFSGSGSGTDFTLTISSLQPEDFAVYFCSQSTHVPYTFGQGTKVEIK

SEQ ID NO: 84 - protein, 112 aa, synthetic construct
  source 1..112: note; note (original language) = 人源化抗体hu2117-HK-Mu03的VL
DVQMTQSPSSLSASVGDRVTITCRSSQSLVHSNGNTYLHWYQQKPGKAPKLLIYKVSNRFSGVPSRFSGSGSGTDFTLTISSLQPEDFATYFCSQSTHVPYTFGQGTKVEIK

SEQ ID NO: 85 - protein, 112 aa, synthetic construct
  source 1..112: note; note (original language) = 人源化抗体hu2117-HK-Mu04的VL
DIQLTQSPSSLSASVGDRVTITCRSSQSLVHSNGNTYLHWYQQKPGKAPKLLIYKVSNRFSGVPSRFSGSGSGTDFTLTISSLQPEDFATYFCSQSTHVPYTFGQGTKVEIK

SEQ ID NO: 86 - protein, 112 aa, synthetic construct
  source 1..112: note; note (original language) = 人源化抗体hu2117-HK-Mu11的VL
DIQMTQSPSSLSASVGDRVTITCRSSQSLVHSNGNTYLHWYQQKPGKAPKLLIYKVSNRDSGVPSRFSGSGSGTDFTLTISSLQPEDFATYFCSQSTHVPYTFGQGTKVEIK

SEQ ID NO: 87 - protein, 112 aa, synthetic construct
  source 1..112: note; note (original language) = 人源化抗体hu2117-HK-Mu12的VL
DIQMTQSPSSLSASVGDRVTITCRSSQSLVHSNGNTYLHWYQQKPGKAPKLLIYKVSNRPSGVPSRFSGSGSGTDFTLTISSLQPEDFATYFCSQSTHVPYTFGQGTKVEIK

SEQ ID NO: 88 - protein, 112 aa, synthetic construct
  source 1..112: note; note (original language) = 人源化抗体hu2117-HK-Mu13的VL
DIQMTQSPSSLSASVGDRVTITCRSSQSLVHSNGNTYLHWYQQKPGKAPKLLIYKVSNRFSGVPSRFSGSGSGTDFTLTISSLQPEDFATYYCSQSTHVPYTFGQGTKVEIK

SEQ ID NO: 89 - protein, 112 aa, synthetic construct
  source 1..112: note; note (original language) = 人源化抗体hu2117-HK-Mu23的VL
DIQMTQSPSSLSASVGDRVTITCRSSQSLVHSNANTYLHWYQQKPGKAPKLLIYKVSNRFSGVPSRFSGSGSGTDFTLTISSLQPEDFATYFCSQSTHVPYTFGQGTKVEIK

SEQ ID NO: 90 - protein, 112 aa, synthetic construct
  source 1..112: note; note (original language) = 人源化抗体hu2117-HK-Mu24的VL
DIQMTQSPSSLSASVGDRVTITCRSSQSLVHSNINTYLHWYQQKPGKAPKLLIYKVSNRFSGVPSRFSGSGSGTDFTLTISSLQPEDFATYFCSQSTHVPYTFGQGTKVEIK

SEQ ID NO: 91 - protein, 112 aa, synthetic construct
  source 1..112: note; note (original language) = 人源化抗体hu2117-HK-Mu25的VL
DIQMTQSPSSLSASVGDRVTITCRSSQSLVHSNSNTYLHWYQQKPGKAPKLLIYKVSNRFSGVPSRFSGSGSGTDFTLTISSLQPEDFATYFCSQSTHVPYTFGQGTKVEIK

SEQ ID NO: 92 - protein, 112 aa, synthetic construct
  source 1..112: note; note (original language) = VL
DIQMTQSPSSLSASVGDRVTITCRSSQSLVHSNRNTYLHWYQQKPGKAPKLLIYKVSNRFSGVPSRFSGSGSGTDFTLTISSLQPEDFATYFCSQSTHVPYTFGQGTKVEIK

SEQ ID NO: 93 - protein, 112 aa, synthetic construct
  source 1..112: note; note (original language) = 人源化抗体hu2117-HK-Mu28的VL
DIQMTQSPSSLSASVGDRVTITCRSSQSLVHSNTNTYLHWYQQKPGKAPKLLIYKVSNRFSGVPSRFSGSGSGTDFTLTISSLQPEDFATYFCSQSTHVPYTFGQGTKVEIK

SEQ ID NO: 94 - protein, 112 aa, synthetic construct
  source 1..112: note; note (original language) = 人源化抗体hu2117-HK-Mu29的VL
DIQMTQSPSSLSASVGDRVTITCRSSQSLLHSNGNTYLHWYQQKPGKAPKLLIYKVSNRFSGVPSRFSGSGSGTDFTLTISSLQPEDFATYFCSQSTHVPYTFGQGTKVEIK

SEQ ID NO: 95 - protein, 112 aa, synthetic construct
  source 1..112: note; note (original language) = 人源化抗体hu2117-HK-Mu32的VL
DIQMTQSPSSLSASVGDRVTITCRSSQSLVSSNGNTYLHWYQQKPGKAPKLLIYKVSNRFSGVPSRFSGSGSGTDFTLTISSLQPEDFATYFCSQSTHVPYTFGQGTKVEIK

SEQ ID NO: 96 - protein, 112 aa, synthetic construct
  source 1..112: note; note (original language) = 人源化抗体hu2117-HK-Mu34的VL
DIQMTQSPSSLSASVGDRVTITCRSSQSLVHSNGNTYLHWYQQKPGKAPKLLIYKVSNRFSGVPSRFSGSGSGTDFTLTISSLQPEDFATYFCQQSTHVPYTFGQGTKVEIK

SEQ ID NO: 97 - protein, 112 aa, synthetic construct
  source 1..112: note; note (original language) = 人源化抗体hu2117-HK-Mu37的VL
DIQMTQSPSSLSASVGDRVTITCRSSQSLVHSNGNTYLHWYQQKPGKAPKLLIYKVSNRFSGVPSRFSGSGSGTDFTLTISSLQPEDFATYFCSQSTHVPWTFGQGTKVEIK

SEQ ID NO: 98 - protein, 5 aa, Mus musculus
DYSMH

SEQ ID NO: 99 - protein, 5 aa, synthetic construct
  source 1..5: note; note (original language) = 人源化抗体2126-Hu-H24的HCDR1
DYAMH

SEQ ID NO: 100 - protein, 17 aa, Mus musculus
WINTETGEPTYADDFKG

SEQ ID NO: 101 - protein, 17 aa, synthetic construct
  source 1..17: note; note (original language) = 人源化抗体2126-Hu-H25的HCDR2
WINTNTGEPTYADDFKG

SEQ ID NO: 102 - protein, 17 aa, synthetic construct
  source 1..17: note; note (original language) = 人源化抗体2126-Hu-H27，7172b-Mu10至Mu19的HCDR2
WINTGTGEPTYADDFKG

SEQ ID NO: 103 - protein, 17 aa, synthetic construct
  source 1..17: note; note (original language) = 人源化抗体2126-Hu-H28的HCDR2
WINTYTGEPTYADDFKG

SEQ ID NO: 104 - protein, 17 aa, synthetic construct
  source 1..17: note; note (original language) = 人源化抗体2126-Hu-H29的HCDR2
WINTITGEPTYADDFKG

SEQ ID NO: 105 - protein, 17 aa, synthetic construct
  source 1..17: note; note (original language) = 人源化抗体2126-Hu-H31的HCDR2
WINTETGDPTYADDFKG

SEQ ID NO: 106 - protein, 17 aa, synthetic construct
  source 1..17: note; note (original language) = 人源化抗体2126-Hu-H32的HCDR2
WINTETGSPTYADDFKG

SEQ ID NO: 107 - protein, 17 aa, synthetic construct
  source 1..17: note; note (original language) = 人源化抗体2126-Hu-H33的HCDR2
WINTETGEPTYADKFKG

SEQ ID NO: 108 - protein, 17 aa, synthetic construct
  source 1..17: note; note (original language) = 人源化抗体2126-Hu-H34的HCDR2
WINTETGEPTYADNFKG

SEQ ID NO: 109 - protein, 17 aa, synthetic construct
  source 1..17: note; note (original language) = 人源化抗体2126-Hu-H35的HCDR2
WINTETGEPTYADDVKG

SEQ ID NO: 110 - protein, 10 aa, Mus musculus
VGRYDYAMDY

SEQ ID NO: 111 - protein, 10 aa, synthetic construct
  source 1..10: note; note (original language) = 人源化抗体2126-Hu-H50的HCDR3
VGYYDYAMDY

SEQ ID NO: 112 - protein, 10 aa, synthetic construct
  source 1..10: note; note (original language) = 人源化抗体2126-Hu-H54的HCDR3
VGRGDYAMDY

SEQ ID NO: 113 - protein, 10 aa, synthetic construct
  source 1..10: note; note (original language) = 人源化抗体2126-Hu-H59的HCDR3
VGRYSYAMDY

SEQ ID NO: 114 - protein, 11 aa, Mus musculus
KASQDVYTAVA

SEQ ID NO: 115 - protein, 11 aa, synthetic construct
  source 1..11: note; note (original language) = 人源化抗体2126-Hu-L02，以及7172b-Mu10至Mu19的LCDR1
RASQDVYTAVA

SEQ ID NO: 116 - protein, 7 aa, Mus musculus
SASYRYT

SEQ ID NO: 117 - protein, 7 aa, synthetic construct
  source 1..7: note; note (original language) = 人源化抗体2126-Hu-L06的LCDR2
AASYRYT

SEQ ID NO: 118 - protein, 7 aa, synthetic construct
  source 1..7: note; note (original language) = 人源化抗体2126-Hu-L07的LCDR2
SASDRYT

SEQ ID NO: 119 - protein, 7 aa, synthetic construct
  source 1..7: note; note (original language) = 人源化抗体2126-Hu-L08的LCDR2
SASERYT

SEQ ID NO: 120 - protein, 7 aa, synthetic construct
  source 1..7: note; note (original language) = 人源化抗体2126-Hu-L09的LCDR2
SASKRYT

SEQ ID NO: 121 - protein, 7 aa, synthetic construct
  source 1..7: note; note (original language) = 人源化抗体2126-Hu-L10的LCDR2
SASNRYT

SEQ ID NO: 122 - protein, 7 aa, synthetic construct
  source 1..7: note; note (original language) = 人源化抗体2126-Hu-L11的LCDR2
SASQRYT

SEQ ID NO: 123 - protein, 7 aa, synthetic construct
  source 1..7: note; note (original language) = 人源化抗体2126-Hu-L12的LCDR2
SASSRYT

SEQ ID NO: 124 - protein, 7 aa, synthetic construct
  source 1..7: note; note (original language) = 人源化抗体2126-Hu-L13的LCDR2
SASTRYT

SEQ ID NO: 125 - protein, 7 aa, synthetic construct
  source 1..7: note; note (original language) = 人源化抗体2126-Hu-L14的LCDR2
SASYRAT

SEQ ID NO: 126 - protein, 7 aa, synthetic construct
  source 1..7: note; note (original language) = 人源化抗体2126-Hu-L15的LCDR2
SASYRET

SEQ ID NO: 127 - protein, 7 aa, synthetic construct
  source 1..7: note; note (original language) = 人源化抗体2126-Hu-L16的LCDR2
SASYRPT

SEQ ID NO: 128 - protein, 7 aa, synthetic construct
  source 1..7: note; note (original language) = 人源化抗体2126-Hu-L17的LCDR2
SASYRQT

SEQ ID NO: 129 - protein, 7 aa, synthetic construct
  source 1..7: note; note (original language) = 人源化抗体7172b-Mu10的LCDR2
AASSRPT

SEQ ID NO: 130 - protein, 7 aa, synthetic construct
  source 1..7: note; note (original language) = 人源化抗体7172b-Mu11的LCDR2
DASSRPT

SEQ ID NO: 131 - protein, 7 aa, synthetic construct
  source 1..7: note; note (original language) = 人源化抗体7172b-Mu12的LCDR2
EASSRPT

SEQ ID NO: 132 - protein, 7 aa, synthetic construct
  source 1..7: note; note (original language) = 人源化抗体7172b-Mu13的LCDR2
KASSRPT

SEQ ID NO: 133 - protein, 7 aa, synthetic construct
  source 1..7: note; note (original language) = 人源化抗体7172b-Mu14的LCDR2
LASSRPT

SEQ ID NO: 134 - protein, 7 aa, synthetic construct
  source 1..7: note; note (original language) = 人源化抗体7172b-Mu15的LCDR2
QASSRPT

SEQ ID NO: 135 - protein, 7 aa, synthetic construct
  source 1..7: note; note (original language) = 人源化抗体7172b-Mu16的LCDR2
RASSRPT

SEQ ID NO: 136 - protein, 7 aa, synthetic construct
  source 1..7: note; note (original language) = 人源化抗体7172b-Mu17的LCDR2
SASSRPT

SEQ ID NO: 137 - protein, 7 aa, synthetic construct
  source 1..7: note; note (original language) = 人源化抗体7172b-Mu18的LCDR2
WASSRPT

SEQ ID NO: 138 - protein, 7 aa, synthetic construct
  source 1..7: note; note (original language) = 人源化抗体7172b-Mu19的LCDR2
YASSRPT

SEQ ID NO: 139 - protein, 9 aa, Mus musculus
QQHYSTPPT

SEQ ID NO: 140 - protein, 9 aa, synthetic construct
  source 1..9: note; note (original language) = 人源化抗体2126-Hu-L18的LCDR3
QQSYSTPPT

SEQ ID NO: 141 - protein, 9 aa, synthetic construct
  source 1..9: note; note (original language) = 人源化抗体2126-Hu-L19的LCDR3
QQAYSTPPT

SEQ ID NO: 142 - protein, 9 aa, synthetic construct
  source 1..9: note; note (original language) = 人源化抗体2126-Hu-L21，以及7172b-Mu10至Mu19的LCDR3
QQYYSTPPT

SEQ ID NO: 143 - protein, 119 aa, synthetic construct
  source 1..119: note; note (original language) = 人源化抗体hu2126-H2K1，2126-Hu-L02、L05至L19、L21的VH
QVQLVQSGSELKKPGASVKVSCKASGYTFTDYSMHWVRQAPGQGLEWMGWINTETGEPTYADDFKGRFVFSLDTSVSTAYLQISSLKAEDTAVYFCVRVGRYDYAMDYWGQGTTVTVSS

SEQ ID NO: 144 - protein, 119 aa, synthetic construct
  source 1..119: note; note (original language) = 人源化抗体2126-Hu-H22的VH
QVQLVQSGGELKKPGASVKVSCKASGYTFTDYSMHWVRQAPGQGLEWMGWINTETGEPTYADDFKGRFVFSLDTSVSTAYLQISSLKAEDTAVYFCVRVGRYDYAMDYWGQGTTVTVSS

SEQ ID NO: 145 - protein, 119 aa, synthetic construct
  source 1..119: note; note (original language) = 人源化抗体2126-Hu-H23的VH
QVQLVQSGSELKKPGASLKVSCKASGYTFTDYSMHWVRQAPGQGLEWMGWINTETGEPTYADDFKGRFVFSLDTSVSTAYLQISSLKAEDTAVYFCVRVGRYDYAMDYWGQGTTVTVSS

SEQ ID NO: 146 - protein, 119 aa, synthetic construct
  source 1..119: note; note (original language) = 人源化抗体2126-Hu-H24的VH
QVQLVQSGSELKKPGASVKVSCKASGYTFTDYAMHWVRQAPGQGLEWMGWINTETGEPTYADDFKGRFVFSLDTSVSTAYLQISSLKAEDTAVYFCVRVGRYDYAMDYWGQGTTVTVSS

SEQ ID NO: 147 - protein, 119 aa, synthetic construct
  source 1..119: note; note (original language) = 人源化抗体2126-Hu-H25的VH
QVQLVQSGSELKKPGASVKVSCKASGYTFTDYSMHWVRQAPGQGLEWMGWINTNTGEPTYADDFKGRFVFSLDTSVSTAYLQISSLKAEDTAVYFCVRVGRYDYAMDYWGQGTTVTVSS

SEQ ID NO: 148 - protein, 119 aa, synthetic construct
  source 1..119: note; note (original language) = 人源化抗体2126-Hu-H27的VH
QVQLVQSGSELKKPGASVKVSCKASGYTFTDYSMHWVRQAPGQGLEWMGWINTGTGEPTYADDFKGRFVFSLDTSVSTAYLQISSLKAEDTAVYFCVRVGRYDYAMDYWGQGTTVTVSS

SEQ ID NO: 149 - protein, 119 aa, synthetic construct
  source 1..119: note; note (original language) = 人源化抗体2126-Hu-H28的VH
QVQLVQSGSELKKPGASVKVSCKASGYTFTDYSMHWVRQAPGQGLEWMGWINTYTGEPTYADDFKGRFVFSLDTSVSTAYLQISSLKAEDTAVYFCVRVGRYDYAMDYWGQGTTVTVSS

SEQ ID NO: 150 - protein, 119 aa, synthetic construct
  source 1..119: note; note (original language) = 人源化抗体2126-Hu-H29的VH
QVQLVQSGSELKKPGASVKVSCKASGYTFTDYSMHWVRQAPGQGLEWMGWINTITGEPTYADDFKGRFVFSLDTSVSTAYLQISSLKAEDTAVYFCVRVGRYDYAMDYWGQGTTVTVSS

SEQ ID NO: 151 - protein, 119 aa, synthetic construct
  source 1..119: note; note (original language) = 人源化抗体2126-Hu-H31的VH
QVQLVQSGSELKKPGASVKVSCKASGYTFTDYSMHWVRQAPGQGLEWMGWINTETGDPTYADDFKGRFVFSLDTSVSTAYLQISSLKAEDTAVYFCVRVGRYDYAMDYWGQGTTVTVSS

SEQ ID NO: 152 - protein, 119 aa, synthetic construct
  source 1..119: note; note (original language) = 人源化抗体2126-Hu-H32的VH
QVQLVQSGSELKKPGASVKVSCKASGYTFTDYSMHWVRQAPGQGLEWMGWINTETGSPTYADDFKGRFVFSLDTSVSTAYLQISSLKAEDTAVYFCVRVGRYDYAMDYWGQGTTVTVSS

SEQ ID NO: 153 - protein, 119 aa, synthetic construct
  source 1..119: note; note (original language) = 人源化抗体2126-Hu-H33的VH
QVQLVQSGSELKKPGASVKVSCKASGYTFTDYSMHWVRQAPGQGLEWMGWINTETGEPTYADKFKGRFVFSLDTSVSTAYLQISSLKAEDTAVYFCVRVGRYDYAMDYWGQGTTVTVSS

SEQ ID NO: 154 - protein, 119 aa, synthetic construct
  source 1..119: note; note (original language) = 人源化抗体2126-Hu-H34的VH
QVQLVQSGSELKKPGASVKVSCKASGYTFTDYSMHWVRQAPGQGLEWMGWINTETGEPTYADNFKGRFVFSLDTSVSTAYLQISSLKAEDTAVYFCVRVGRYDYAMDYWGQGTTVTVSS

SEQ ID NO: 155 - protein, 119 aa, synthetic construct
  source 1..119: note; note (original language) = 人源化抗体2126-Hu-H35的VH
QVQLVQSGSELKKPGASVKVSCKASGYTFTDYSMHWVRQAPGQGLEWMGWINTETGEPTYADDVKGRFVFSLDTSVSTAYLQISSLKAEDTAVYFCVRVGRYDYAMDYWGQGTTVTVSS

SEQ ID NO: 156 - protein, 119 aa, synthetic construct
  source 1..119: note; note (original language) = 人源化抗体2126-Hu-H36的VH
QVQLVQSGSELKKPGASVKVSCKASGYTFTDYSMHWVRQAPGQGLEWMGWINTETGEPTYADDFKGRFTFSLDTSVSTAYLQISSLKAEDTAVYFCVRVGRYDYAMDYWGQGTTVTVSS

SEQ ID NO: 157 - protein, 119 aa, synthetic construct
  source 1..119: note; note (original language) = 人源化抗体2126-Hu-H37的VH
QVQLVQSGSELKKPGASVKVSCKASGYTFTDYSMHWVRQAPGQGLEWMGWINTETGEPTYADDFKGRFSFSLDTSVSTAYLQISSLKAEDTAVYFCVRVGRYDYAMDYWGQGTTVTVSS

SEQ ID NO: 158 - protein, 119 aa, synthetic construct
  source 1..119: note; note (original language) = 人源化抗体2126-Hu-H38的VH
QVQLVQSGSELKKPGASVKVSCKASGYTFTDYSMHWVRQAPGQGLEWMGWINTETGEPTYADDFKGRFVISLDTSVSTAYLQISSLKAEDTAVYFCVRVGRYDYAMDYWGQGTTVTVSS

SEQ ID NO: 159 - protein, 119 aa, synthetic construct
  source 1..119: note; note (original language) = 人源化抗体2126-Hu-H39的VH
QVQLVQSGSELKKPGASVKVSCKASGYTFTDYSMHWVRQAPGQGLEWMGWINTETGEPTYADDFKGRFVFSVDTSVSTAYLQISSLKAEDTAVYFCVRVGRYDYAMDYWGQGTTVTVSS

SEQ ID NO: 160 - protein, 119 aa, synthetic construct
  source 1..119: note; note (original language) = 人源化抗体2126-Hu-H40的VH
QVQLVQSGSELKKPGASVKVSCKASGYTFTDYSMHWVRQAPGQGLEWMGWINTETGEPTYADDFKGRFVFSRDTSVSTAYLQISSLKAEDTAVYFCVRVGRYDYAMDYWGQGTTVTVSS

SEQ ID NO: 161 - protein, 119 aa, synthetic construct
  source 1..119: note; note (original language) = 人源化抗体2126-Hu-H42的VH
QVQLVQSGSELKKPGASVKVSCKASGYTFTDYSMHWVRQAPGQGLEWMGWINTETGEPTYADDFKGRFVFSLDTSKSTAYLQISSLKAEDTAVYFCVRVGRYDYAMDYWGQGTTVTVSS

SEQ ID NO: 162 - protein, 119 aa, synthetic construct
  source 1..119: note; note (original language) = 人源化抗体2126-Hu-H43的VH
QVQLVQSGSELKKPGASVKVSCKASGYTFTDYSMHWVRQAPGQGLEWMGWINTETGEPTYADDFKGRFVFSLDTSTSTAYLQISSLKAEDTAVYFCVRVGRYDYAMDYWGQGTTVTVSS

SEQ ID NO: 163 - protein, 119 aa, synthetic construct
  source 1..119: note; note (original language) = 人源化抗体2126-Hu-H44的VH
QVQLVQSGSELKKPGASVKVSCKASGYTFTDYSMHWVRQAPGQGLEWMGWINTETGEPTYADDFKGRFVFSLDTSVSTAYLQLSSLKAEDTAVYFCVRVGRYDYAMDYWGQGTTVTVSS

SEQ ID NO: 164 - protein, 119 aa, synthetic construct
  source 1..119: note; note (original language) = 人源化抗体2126-Hu-H45的VH
QVQLVQSGSELKKPGASVKVSCKASGYTFTDYSMHWVRQAPGQGLEWMGWINTETGEPTYADDFKGRFVFSLDTSVSTAYLQMSSLKAEDTAVYFCVRVGRYDYAMDYWGQGTTVTVSS

SEQ ID NO: 165 - protein, 119 aa, synthetic construct
  source 1..119: note; note (original language) = 人源化抗体2126-Hu-H46的VH
QVQLVQSGSELKKPGASVKVSCKASGYTFTDYSMHWVRQAPGQGLEWMGWINTETGEPTYADDFKGRFVFSLDTSVSTAYLQISSLKAEDTAVYYCVRVGRYDYAMDYWGQGTTVTVSS

SEQ ID NO: 166 - protein, 119 aa, synthetic construct
  source 1..119: note; note (original language) = 人源化抗体2126-Hu-H50的VH
QVQLVQSGSELKKPGASVKVSCKASGYTFTDYSMHWVRQAPGQGLEWMGWINTETGEPTYADDFKGRFVFSLDTSVSTAYLQISSLKAEDTAVYFCVRVGYYDYAMDYWGQGTTVTVSS

SEQ ID NO: 167 - protein, 119 aa, synthetic construct
  source 1..119: note; note (original language) = 人源化抗体2126-Hu-H54的VH
QVQLVQSGSELKKPGASVKVSCKASGYTFTDYSMHWVRQAPGQGLEWMGWINTETGEPTYADDFKGRFVFSLDTSVSTAYLQISSLKAEDTAVYFCVRVGRGDYAMDYWGQGTTVTVSS

SEQ ID NO: 168 - protein, 119 aa, synthetic construct
  source 1..119: note; note (original language) = 人源化抗体2126-Hu-H59的VH
QVQLVQSGSELKKPGASVKVSCKASGYTFTDYSMHWVRQAPGQGLEWMGWINTETGEPTYADDFKGRFVFSLDTSVSTAYLQISSLKAEDTAVYFCVRVGRYSYAMDYWGQGTTVTVSS

SEQ ID NO: 169 - protein, 119 aa, synthetic construct
  source 1..119: note; note (original language) = 人源化抗体7172b-Mu10至Mu19的VH
QVQLVQSGSELKKPGASVKVSCKASGYTFTDYSMHWVRQAPGQGLEWMGWINTGTGEPTYADDFKGRFTISRDTSKSTAYLQISSLKAEDTAVYYCVRVGRYDYAMDYWGQGTTVTVSS

SEQ ID NO: 170 - protein, 119 aa, synthetic construct
  source 1..119: note; note (original language) = 人源化抗体Hu2126_H1的VH
QVQLQESGPGLVKPSETLSLTCTASGYTFTDYSMHWVRQPPGKGLEWMGWINTETGEPTYADDFKGRFTFSLDTSKNQASLKLSSVTAADTAVYFCVRVGRYDYAMDYWGQGTTVTVSS

SEQ ID NO: 171 - protein, 107 aa, synthetic construct
  source 1..107: note; note (original language) = VL
DIQMTQSPSSLSASVGDRVTITCKASQDVYTAVAWYQQKPGKAPKLLINSASYRYTGVPSRFSGSGSGTDFTLTISSLQPEDFATYYCQQHYSTPPTFGGGTKVEIK

SEQ ID NO: 172 - protein, 107 aa, synthetic construct
  source 1..107: note; note (original language) = 人源化抗体2126-Hu-L02的VL
DIQMTQSPSSLSASVGDRVTITCRASQDVYTAVAWYQQKPGKAPKLLINSASYRYTGVPSRFSGSGSGTDFTLTISSLQPEDFATYYCQQHYSTPPTFGGGTKVEIK

SEQ ID NO: 173 - protein, 107 aa, synthetic construct
  source 1..107: note; note (original language) = 人源化抗体2126-Hu-L05的VL
DIQMTQSPSSLSASVGDRVTITCKASQDVYTAVAWYQQKPGKAPKLLIYSASYRYTGVPSRFSGSGSGTDFTLTISSLQPEDFATYYCQQHYSTPPTFGGGTKVEIK

SEQ ID NO: 174 - protein, 107 aa, synthetic construct
  source 1..107: note; note (original language) = 人源化抗体2126-Hu-L06的VL
DIQMTQSPSSLSASVGDRVTITCKASQDVYTAVAWYQQKPGKAPKLLINAASYRYTGVPSRFSGSGSGTDFTLTISSLQPEDFATYYCQQHYSTPPTFGGGTKVEIK

SEQ ID NO: 175 - protein, 107 aa, synthetic construct
  source 1..107: note; note (original language) = 人源化抗体2126-Hu-L07的VL
DIQMTQSPSSLSASVGDRVTITCKASQDVYTAVAWYQQKPGKAPKLLINSASDRYTGVPSRFSGSGSGTDFTLTISSLQPEDFATYYCQQHYSTPPTFGGGTKVEIK

SEQ ID NO: 176 - protein, 107 aa, synthetic construct
  source 1..107: note; note (original language) = 人源化抗体2126-Hu-L08的VL
DIQMTQSPSSLSASVGDRVTITCKASQDVYTAVAWYQQKPGKAPKLLINSASERYTGVPSRFSGSGSGTDFTLTISSLQPEDFATYYCQQHYSTPPTFGGGTKVEIK

SEQ ID NO: 177 - protein, 107 aa, synthetic construct
  source 1..107: note; note (original language) = 人源化抗体2126-Hu-L09的VL
DIQMTQSPSSLSASVGDRVTITCKASQDVYTAVAWYQQKPGKAPKLLINSASKRYTGVPSRFSGSGSGTDFTLTISSLQPEDFATYYCQQHYSTPPTFGGGTKVEIK

SEQ ID NO: 178 - protein, 107 aa, synthetic construct
  source 1..107: note; note (original language) = 人源化抗体2126-Hu-L10的VL
DIQMTQSPSSLSASVGDRVTITCKASQDVYTAVAWYQQKPGKAPKLLINSASNRYTGVPSRFSGSGSGTDFTLTISSLQPEDFATYYCQQHYSTPPTFGGGTKVEIK

SEQ ID NO: 179 - protein, 107 aa, synthetic construct
  source 1..107: note; note (original language) = 人源化抗体2126-Hu-L11的VL
DIQMTQSPSSLSASVGDRVTITCKASQDVYTAVAWYQQKPGKAPKLLINSASQRYTGVPSRFSGSGSGTDFTLTISSLQPEDFATYYCQQHYSTPPTFGGGTKVEIK

SEQ ID NO: 180 - protein, 107 aa, synthetic construct
  source 1..107: note; note (original language) = 人源化抗体2126-Hu-L12的VL
DIQMTQSPSSLSASVGDRVTITCKASQDVYTAVAWYQQKPGKAPKLLINSASSRYTGVPSRFSGSGSGTDFTLTISSLQPEDFATYYCQQHYSTPPTFGGGTKVEIK

SEQ ID NO: 181 - protein, 107 aa, synthetic construct
  source 1..107: note; note (original language) = 人源化抗体2126-Hu-L13的VL
DIQMTQSPSSLSASVGDRVTITCKASQDVYTAVAWYQQKPGKAPKLLINSASTRYTGVPSRFSGSGSGTDFTLTISSLQPEDFATYYCQQHYSTPPTFGGGTKVEIK

SEQ ID NO: 182 - protein, 107 aa, synthetic construct
  source 1..107: note; note (original language) = 人源化抗体2126-Hu-L14的VL
DIQMTQSPSSLSASVGDRVTITCKASQDVYTAVAWYQQKPGKAPKLLINSASYRATGVPSRFSGSGSGTDFTLTISSLQPEDFATYYCQQHYSTPPTFGGGTKVEIK

SEQ ID NO: 183 - protein, 107 aa, synthetic construct
  source 1..107: note; note (original language) = 人源化抗体2126-Hu-L15的VL
DIQMTQSPSSLSASVGDRVTITCKASQDVYTAVAWYQQKPGKAPKLLINSASYRETGVPSRFSGSGSGTDFTLTISSLQPEDFATYYCQQHYSTPPTFGGGTKVEIK

SEQ ID NO: 184 - protein, 107 aa, synthetic construct
  source 1..107: note; note (original language) = 人源化抗体2126-Hu-L16的VL
DIQMTQSPSSLSASVGDRVTITCKASQDVYTAVAWYQQKPGKAPKLLINSASYRPTGVPSRFSGSGSGTDFTLTISSLQPEDFATYYCQQHYSTPPTFGGGTKVEIK

SEQ ID NO: 185 - protein, 107 aa, synthetic construct
  source 1..107: note; note (original language) = 人源化抗体2126-Hu-L17的VL
DIQMTQSPSSLSASVGDRVTITCKASQDVYTAVAWYQQKPGKAPKLLINSASYRQTGVPSRFSGSGSGTDFTLTISSLQPEDFATYYCQQHYSTPPTFGGGTKVEIK

SEQ ID NO: 186 - protein, 107 aa, synthetic construct
  source 1..107: note; note (original language) = 人源化抗体2126-Hu-L18的VL
DIQMTQSPSSLSASVGDRVTITCKASQDVYTAVAWYQQKPGKAPKLLINSASYRYTGVPSRFSGSGSGTDFTLTISSLQPEDFATYYCQQSYSTPPTFGGGTKVEIK

SEQ ID NO: 187 - protein, 107 aa, synthetic construct
  source 1..107: note; note (original language) = 人源化抗体2126-Hu-L19的VL
DIQMTQSPSSLSASVGDRVTITCKASQDVYTAVAWYQQKPGKAPKLLINSASYRYTGVPSRFSGSGSGTDFTLTISSLQPEDFATYYCQQAYSTPPTFGGGTKVEIK

SEQ ID NO: 188 - protein, 107 aa, synthetic construct
  source 1..107: note; note (original language) = 人源化抗体2126-Hu-L21的VL
DIQMTQSPSSLSASVGDRVTITCKASQDVYTAVAWYQQKPGKAPKLLINSASYRYTGVPSRFSGSGSGTDFTLTISSLQPEDFATYYCQQYYSTPPTFGGGTKVEIK

SEQ ID NO: 189 - protein, 107 aa, synthetic construct
  source 1..107: note; note (original language) = 人源化抗体7172b-Mu10的VL
DIQMTQSPSSLSASVGDRVTITCRASQDVYTAVAWYQQKPGKAPKLLINAASSRPTGVPSRFSGSGSGTDFTLTISSLQPEDFATYYCQQYYSTPPTFGGGTKVEIK

SEQ ID NO: 190 - protein, 107 aa, synthetic construct
  source 1..107: note; note (original language) = 人源化抗体7172b-Mu11的VL
DIQMTQSPSSLSASVGDRVTITCRASQDVYTAVAWYQQKPGKAPKLLINDASSRPTGVPSRFSGSGSGTDFTLTISSLQPEDFATYYCQQYYSTPPTFGGGTKVEIK

SEQ ID NO: 191 - protein, 107 aa, synthetic construct
  source 1..107: note; note (original language) = 人源化抗体7172b-Mu12的VL
DIQMTQSPSSLSASVGDRVTITCRASQDVYTAVAWYQQKPGKAPKLLINEASSRPTGVPSRFSGSGSGTDFTLTISSLQPEDFATYYCQQYYSTPPTFGGGTKVEIK

SEQ ID NO: 192 - protein, 107 aa, synthetic construct
  source 1..107: note; note (original language) = 人源化抗体7172b-Mu13的VL
DIQMTQSPSSLSASVGDRVTITCRASQDVYTAVAWYQQKPGKAPKLLINKASSRPTGVPSRFSGSGSGTDFTLTISSLQPEDFATYYCQQYYSTPPTFGGGTKVEIK

SEQ ID NO: 193 - protein, 107 aa, synthetic construct
  source 1..107: note; note (original language) = 人源化抗体7172b-Mu14的VL
DIQMTQSPSSLSASVGDRVTITCRASQDVYTAVAWYQQKPGKAPKLLINLASSRPTGVPSRFSGSGSGTDFTLTISSLQPEDFATYYCQQYYSTPPTFGGGTKVEIK

SEQ ID NO: 194 - protein, 107 aa, synthetic construct
  source 1..107: note; note (original language) = 人源化抗体7172b-Mu15的VL
DIQMTQSPSSLSASVGDRVTITCRASQDVYTAVAWYQQKPGKAPKLLINQASSRPTGVPSRFSGSGSGTDFTLTISSLQPEDFATYYCQQYYSTPPTFGGGTKVEIK

SEQ ID NO: 195 - protein, 107 aa, synthetic construct
  source 1..107: note; note (original language) = 人源化抗体7172b-Mu16的VL
DIQMTQSPSSLSASVGDRVTITCRASQDVYTAVAWYQQKPGKAPKLLINRASSRPTGVPSRFSGSGSGTDFTLTISSLQPEDFATYYCQQYYSTPPTFGGGTKVEIK

SEQ ID NO: 196 - protein, 107 aa, synthetic construct
  source 1..107: note; note (original language) = 人源化抗体7172b-Mu17的VL
DIQMTQSPSSLSASVGDRVTITCRASQDVYTAVAWYQQKPGKAPKLLINSASSRPTGVPSRFSGSGSGTDFTLTISSLQPEDFATYYCQQYYSTPPTFGGGTKVEIK

SEQ ID NO: 197 - protein, 107 aa, synthetic construct
  source 1..107: note; note (original language) = 人源化抗体7172b-Mu18的VL
DIQMTQSPSSLSASVGDRVTITCRASQDVYTAVAWYQQKPGKAPKLLINWASSRPTGVPSRFSGSGSGTDFTLTISSLQPEDFATYYCQQYYSTPPTFGGGTKVEIK

SEQ ID NO: 198 - protein, 107 aa, synthetic construct
  source 1..107: note; note (original language) = 人源化抗体7172b-Mu19的VL
DIQMTQSPSSLSASVGDRVTITCRASQDVYTAVAWYQQKPGKAPKLLINYASSRPTGVPSRFSGSGSGTDFTLTISSLQPEDFATYYCQQYYSTPPTFGGGTKVEIK

SEQ ID NO: 199 - protein, 5 aa, Mus musculus
DYNMD

SEQ ID NO: 200 - protein, 17 aa, Mus musculus
DINPNNGGTIYNQKFKG

SEQ ID NO: 201 - protein, 10 aa, Mus musculus
YGSGYGGFAY

SEQ ID NO: 202 - protein, 12 aa, Mus musculus
SASSSISSNYLH

SEQ ID NO: 203 - protein, 7 aa, Mus musculus
RTSNLAS

SEQ ID NO: 204 - protein, 9 aa, Mus musculus
QQGSSIPRT

SEQ ID NO: 205 - protein, 5 aa, Mus musculus
NYWIE

SEQ ID NO: 206 - protein, 17 aa, Mus musculus
EILPGGDSANYNEIFKG

SEQ ID NO: 207 - protein, 11 aa, Mus musculus
GGGNYPYYFDS

SEQ ID NO: 208 - protein, 11 aa, Mus musculus
KASQDVGTAVA

SEQ ID NO: 209 - protein, 7 aa, Mus musculus
WASTRHT

SEQ ID NO: 210 - protein, 9 aa, Mus musculus
QQYSSYPRT

SEQ ID NO: 211 - protein, 5 aa, Mus musculus
NYWIE

SEQ ID NO: 212 - protein, 17 aa, Mus musculus
EILPGSDTSKNNEIFKG

SEQ ID NO: 213 - protein, 11 aa, Mus musculus
GGNNYPYYFDY

SEQ ID NO: 214 - protein, 11 aa, Mus musculus
KASQDVGTAVA

SEQ ID NO: 215 - protein, 7 aa, Mus musculus
WASTRHT

SEQ ID NO: 216 - protein, 9 aa, Mus musculus
QQYSSYPWT

SEQ ID NO: 217 - protein, 5 aa, synthetic construct
  source 1..5: note; note (original language) = 抗体2117的HCDR1
  VARIANT 1: note; note (original language) = X=S、N或D
XYGMS

SEQ ID NO: 218 - protein, 17 aa, synthetic construct
  source 1..17: note; note (original language) = 抗体2117的HCDR2
  VARIANT 5: note; note (original language) = X=G或S
  VARIANT 7: note; note (original language) = X=S或N
  VARIANT 9: note; note (original language) = X=T或A
  VARIANT 12: note; note (original language) = X=P、A、G或V
  VARIANT 13: note; note (original language) = X=D、E、P、Q或R
  VARIANT 14: note; note (original language) = X=S、K或N
SISGXGXYXKYXXXVKG

SEQ ID NO: 219 - protein, 8 aa, synthetic construct
  source 1..8: note; note (original language) = 抗体2117的HCDR3
  VARIANT 3: note; note (original language) = X=A、I、N、Q、R、S或V
DYXGFFDV

SEQ ID NO: 220 - protein, 16 aa, synthetic construct
  source 1..16: note; note (original language) = 抗体2117的LCDR1
  VARIANT 7: note; note (original language) = X=V或L
  VARIANT 8: note; note (original language) = X=H、S或Y
  VARIANT 11: note; note (original language) = X=G、A、I、S、R或T
RSSQSLXXSNXNTYLH

SEQ ID NO: 221 - protein, 7 aa, synthetic construct
  source 1..7: note; note (original language) = 抗体2117的LCDR2
  VARIANT 6: note; note (original language) = X=F、D或P
KVSNRXS

SEQ ID NO: 222 - protein, 9 aa, synthetic construct
  source 1..9: note; note (original language) = 抗体2117的LCDR3
  VARIANT 1: note; note (original language) = X=S或Q
  VARIANT 8: note; note (original language) = X=Y或W
XQSTHVPXT

SEQ ID NO: 223 - protein, 5 aa, synthetic construct
  source 1..5: note; note (original language) = 抗体2126的HCDR1
  VARIANT 3: note; note (original language) = X=S或A
DYXMH

SEQ ID NO: 224 - protein, 17 aa, synthetic construct
  source 1..17: note; note (original language) = 抗体2126的HCDR2
  VARIANT 5: note; note (original language) = X=E、N、G、Y或I
  VARIANT 8: note; note (original language) = X=E、D或S
  VARIANT 14: note; note (original language) = X=D、K或N
  VARIANT 15: note; note (original language) = X=F或V
WINTXTGXPTYADXXKG

SEQ ID NO: 225 - protein, 10 aa, synthetic construct
  source 1..10: note; note (original language) = 抗体2126的HCDR3
  VARIANT 3: note; note (original language) = X=R或Y
  VARIANT 4: note; note (original language) = X=Y或G
  VARIANT 5: note; note (original language) = X=D或S
VGXXXYAMDY

SEQ ID NO: 226 - protein, 11 aa, synthetic construct
  source 1..11: note; note (original language) = 抗体2126的LCDR1
  VARIANT 1: note; note (original language) = X=K或R
XASQDVYTAVA

SEQ ID NO: 227 - protein, 7 aa, synthetic construct
  source 1..7: note; note (original language) = 抗体2126的LCDR2
  VARIANT 1: note; note (original language) = X=S、A、D、E、K、L、Q、R、W或Y
  VARIANT 4: note; note (original language) = X=Y、D、E、K、N、Q、S或T
  VARIANT 6: note; note (original language) = X=Y、A、E、P或Q
XASXRXT

SEQ ID NO: 228 - protein, 9 aa, synthetic construct
  source 1..9: note; note (original language) = 抗体2126的LCDR3
  VARIANT 3: note; note (original language) = X=H、S、A或Y
QQXYSTPPT

SEQ ID NO: 229 - protein, 5 aa, synthetic construct
  source 1..5: note; note (original language) = 连接子
GGGGS

SEQ ID NO: 230 - protein, 15 aa, synthetic construct
  source 1..15: note; note (original language) = 连接子
GGGGSGGGGSGGGGS

SEQ ID NO: 231 - protein, 330 aa, Homo sapiens
ASTKGPSVFPLAPSSKSTSGGTAALGCLVKDYFPEPVTVSWNSGALTSGVHTFPAVLQSSGLYSLSSVVTVPSSSLGTQTYICNVNHKPSNTKVDKRVEPKSCDKTHTCPPCPAPELLGGPSVFLFPPKPKDTLMISRTPEVTCVVVDVSHEDPEVKFNWYVDGVEVHNAKTKPREEQYNSTYRVVSVLTVLHQDWLNGKEYKCKVSNKALPAPIEKTISKAKGQPREPQVYTLPPSRDELTKNQVSLTCLVKGFYPSDIAVEWESNGQPENNYKTTPPVLDSDGSFFLYSKLTVDKSRWQQGNVFSCSVMHEALHNHYTQKSLSLSPGK

SEQ ID NO: 232 - protein, 232 aa, synthetic construct
  source 1..232: note; note (original language) = 包含TM突变的IgG1 Fc
EPKSCDKTHTCPPCPAPEFEGGPSVFLFPPKPKDTLMISRTPEVTCVVVDVSHEDPEVKFNWYVDGVEVHNAKTKPREEQYNSTYRVVSVLTVLHQDWLNGKEYKCKVSNKALPASIEKTISKAKGQPREPQVYTLPPSRDELTKNQVSLTCLVKGFYPSDIAVEWESNGQPENNYKTTPPVLDSDGSFFLYSKLTVDKSRWQQGNVFSCSVMHEALHNHYTQKSLSLSPGK

SEQ ID NO: 233 - protein, 107 aa, Homo sapiens [sequence omitted]

SEQ ID NO: 234 - protein, 1255 aa, Homo sapiens [sequence omitted]